European Patent Application EP 4 759 330 A1, published June 17, 2026. Title: 抗FRα抗体药物偶联物在治疗疾病中的应用. Applicant: 百奥泰生物制药股份有限公司. The sequence listing filed with the application follows.

SEQUENCE LISTING (22 sequences)

SEQ ID NO: 1 - protein, 5 aa, synthetic construct
GYFMN

SEQ ID NO: 2 - protein, 17 aa, synthetic construct
RIHPYDGDTFYNQNFKD

SEQ ID NO: 3 - protein, 9 aa, synthetic construct
YDGSRAMDY

SEQ ID NO: 4 - protein, 15 aa, synthetic construct
KASQSVSFAGTSLMH

SEQ ID NO: 5 - protein, 7 aa, synthetic construct
RASNLEA

SEQ ID NO: 6 - protein, 9 aa, synthetic construct
QQSREYPYT

SEQ ID NO: 7 - protein, 118 aa, synthetic construct
QVQLVQSGVEVKKPGASVKVSCKASGYSFTGYFMNWVRQAPGQGLEWIGRIHPYDGDTFYNQNFKDKATLTVDKSTTTAYMELKSLQFDDTAVYYCTRYDGSRAMDYWGQGTTVTVSS

SEQ ID NO: 8 - protein, 111 aa, synthetic construct
EIVLTQSPATLSLSPGERATLSCKASQSVSFAGTSLMHWYQQKPGQAPRLLIYRASNLEAGVPARFSGSGSKTDFTLTISSLEPEDFAVYYCQQSREYPYTFGGGTKVEIK

SEQ ID NO: 9 - protein, 330 aa, synthetic construct [sequence omitted]

SEQ ID NO: 10 - protein, 107 aa, synthetic construct [sequence omitted]

SEQ ID NO: 11 - protein, 448 aa, synthetic construct
QVQLVQSGVEVKKPGASVKVSCKASGYSFTGYFMNWVRQAPGQGLEWIGRIHPYDGDTFYNQNFKDKATLTVDKSTTTAYMELKSLQFDDTAVYYCTRYDGSRAMDYWGQGTTVTVSSASTKGPSVFPLAPSSKSTSGGTAALGCLVKDYFPEPVTVSWNSGALTSGVHTFPAVLQSSGLYSLSSVVTVPSSSLGTQTYICNVNHKPSNTKVDKKVEPKSCDKTHTCPPCPAPELLGGPSVFLFPPKPKDTLMISRTPEVTCVVVDVSHEDPEVKFNWYVDGVEVHNAKTKPREEQYNSTYRVVSVLTVLHQDWLNGKEYKCKVSNKALPAPIEKTISKAKGQPREPQVYTLPPSRDELTKNQVSLTCLVKGFYPSDIAVEWESNGQPENNYKTTPPVLDSDGSFFLYSKLTVDKSRWQQGNVFSCSVMHEALHNHYTQKSLSLSPGK

SEQ ID NO: 12 - DNA, 1347 bp, synthetic construct
  source 1..1347: mol_type = other DNA
caggtgcagctggtgcagtccggcgtggaggtgaagaagcccggcgccagcgtgaaggtgagctgcaaggcctccggctactccttcaccggctacttcatgaactgggtgaggcaggcccccggccagggactggaatggatcggcagaatccacccctacgacggcgacaccttttacaatcagaacttcaaggataaggccaccctgaccgtggataagtccaccaccaccgcctacatggagctgaagtccctgcagtttgacgataccgccgtgtactactgtaccagatacgacggctccagagccatggactactggggccagggcaccaccgtgaccgtgtcctccgccagcaccaagggcccatcggtcttccccctggcaccctcctccaagagcacctctgggggcacagcggccctgggctgcctggtcaaggactacttccccgaaccggtgacggtgtcgtggaactcaggcgccctgaccagcggcgtgcacaccttcccggctgtcctacagtcctcaggactctactccctcagcagcgtggtgaccgtgccctccagcagcttgggcacccagacctacatctgcaacgtgaatcacaagcccagcaacaccaaggtggacaagaaagttgagcccaaatcttgtgacaaaactcacacatgcccaccgtgcccagcacctgaactcctggggggaccgtcagtcttcctcttccccccaaaacccaaggacaccctcatgatctcccggacccctgaggtcacatgcgtggtggtggacgtgagccacgaagaccctgaggtcaagttcaactggtacgtggacggcgtggaggtgcataatgccaagacaaagccgcgggaggagcagtacaacagcacgtaccgtgtggtcagcgtcctcaccgtcctgcaccaggactggctgaatggcaaggagtacaagtgcaaggtctccaacaaagccctcccagcccccatcgagaaaaccatctccaaagccaaagggcagccccgagaaccacaggtgtacaccctgcccccatcccgggatgagctgaccaagaaccaggtcagcctgacctgcctggtcaaaggcttctatcccagcgacatcgccgtggagtgggagagcaatgggcagccggagaacaactacaagaccacgcctcccgtgctggactccgacggctccttcttcctctacagcaagctcaccgtggacaagagcaggtggcagcaggggaacgtcttctcatgctccgtgatgcatgaggctctgcacaaccactacacgcagaagagcctctccctgtctccgggtaaatga

SEQ ID NO: 13 - protein, 218 aa, synthetic construct
EIVLTQSPATLSLSPGERATLSCKASQSVSFAGTSLMHWYQQKPGQAPRLLIYRASNLEAGVPARFSGSGSKTDFTLTISSLEPEDFAVYYCQQSREYPYTFGGGTKVEIKRTVAAPSVFIFPPSDEQLKSGTASVVCLLNNFYPREAKVQWKVDNALQSGNSQESVTEQDSKDSTYSLSSTLTLSKADYEKHKVYACEVTHQGLSSPVTKSFNRGEC

SEQ ID NO: 14 - DNA, 657 bp, synthetic construct
  source 1..657: mol_type = other DNA
gagatcgtgctgacccagtcccccgccaccctgagcctgagcccaggagagagggccaccctgtcctgcaaggcctcccagagcgtgagctttgccggcaccagcctgatgcactggtatcaacagaagcccggccaggcccctaggctgctgatctacagagccagcaacctggaggccggcgtgcctgctaggttttccggcagcggctccaagaccgatttcaccctgaccatcagcagcctggagcctgaggattttgccgtgtactactgccagcagtccagggagtacccctacaccttcggcggcggcaccaaggtggagatcaagcgtacggtggctgcaccatctgtcttcatcttcccgccatctgatgagcagttgaaatctggaactgcctctgttgtgtgcctgctgaataacttctatcccagagaggccaaagtacagtggaaggtggataacgccctccaatcgggtaactcccaggagagtgtcacagagcaggacagcaaggacagcacctacagcctcagcagcaccctgacgctgagcaaagcagactacgagaaacacaaagtctacgcctgcgaagtcacccatcagggcctgagctcgcccgtcacaaagagcttcaacaggggagagtgttga

SEQ ID NO: 15 - protein, 30 aa, synthetic construct
QVQLVQSGVEVKKPGASVKVSCKASGYSFT

SEQ ID NO: 16 - protein, 14 aa, synthetic construct
WVRQAPGQGLEWIG

SEQ ID NO: 17 - protein, 32 aa, synthetic construct
KATLTVDKSTTTAYMELKSLQFDDTAVYYCTR

SEQ ID NO: 18 - protein, 11 aa, synthetic construct
WGQGTTVTVSS

SEQ ID NO: 19 - protein, 23 aa, synthetic construct
EIVLTQSPATLSLSPGERATLSC

SEQ ID NO: 20 - protein, 15 aa, synthetic construct
WYQQKPGQAPRLLIY

SEQ ID NO: 21 - protein, 32 aa, synthetic construct
GVPARFSGSGSKTDFTLTISSLEPEDFAVYYC

SEQ ID NO: 22 - protein, 10 aa, synthetic construct
FGGGTKVEIK